European Patent Specification EP 3 157 564 B1, published April 2, 2025. Title: INTERFERON ALPHA AND OMEGA ANTIBODY ANTAGONISTS. Applicant: JANSSEN BIOTECH, INC. CHI, ELLEN CONNOR, JUDITH HUANG, CHICHI JORDAN, JARRAT LIN-SCHMIDT, XIEFAN LUO, JINQUAN LU, LU MARTINEZ, CHRISTIAN OBMOLOVA, GALINA SWANSON, RONALD. Application To Be Assigned. The sequence listing filed with the application follows.

SEQUENCE LISTING (162 sequences)

SEQ ID NO: 1 - protein, 172 aa, Homo sapiens
CDLPQNHGLLSRNTLVLLHQMRRISPFLCLKDRRDFRFPQEMVKGSQLQKAHVMSVLHEMLQQIFSLFHTERSSAAWNMTLLDQLHTGLHQQLQHLETCLLQVVGEGESAGAISSPALTLRRYFQGIRVYLKEKKYSDCAWEVVRMEIMKSLFLSTNMQERLRSKDRDLGSS

SEQ ID NO: 2 - protein, 172 aa, Homo sapiens
CDLPQNHGLLSRNTLVLLHQMRRISPFLCLKDRRDFRFPQEMVKGSQLQKAHVMSVLHEMLQQIFSLFHTERSSAAWNMELLDQLHTGLHQQLQHLETCLLQVVGEGESAGAISSPALTLRRYFQGIRVYLKEKKYSDCAWEVVRMEIMKSLFLSTNMQERLRSKDRDLGSS

SEQ ID NO: 3 - protein, 177 aa, Pan troglodytes
CDLPQNHGLLSRNTLVLLHQMRRISPFLCLKDRRDFRFPQEMVKGSQLQKAQVMSVLHEMLQQIFSLFHTERSSAAWNMTLLDQLHTGLHQQLQHLETCLLQVMGEGESAGAISSPALTLRRYFQGIRVYLKEKKYSDCAWEVVRMEIMKSLFLSTNMQERLRSKDRDLGSSRNDSH

SEQ ID NO: 4 - protein, 172 aa, Macaca fascicularis
CDLPQNHGLLSRNTLVLLHQMRRISPFLCLKDRRDFRFPQEMVEGSQLQKAQVMSVLHEMLQQIFSLFHTEHSSAAWNTTLLDHLHTGLHRQLEHLETCLVQVMREGESAGAIRSPALTLRRYFQGIRVYLKEKKYSDCAWVVVRMEIMKSLFLSTNMQERLKSKDGDLGSS

SEQ ID NO: 5 - protein, 165 aa, Homo sapiens
CDLPQTHSLGSRRTLMLLAQMRKISLFSCLKDRHDFGFPQEEFGNQFQKAETIPVLHEMIQQIFNLFSTKDSSAAWDETLLDKFYTELYQQLNDLEACVIQGVGVTETPLMKEDSILAVRKYFQRITLYLKEKKYSPCAWEVVRAEIMRSFSLSTNLQESLRSKE

SEQ ID NO: 6 - protein, 166 aa, Homo sapiens
CDLPQTHSLGNRRALILLAQMRRISPFSCLKDRHDFEFPQEEFDDKQFQKAQAISVLHEMIQQTFNLFSTKDSSAALDETLLDEFYIELDQQLNDLESCVMQEVGVIESPLMYEDSILAVRKYFQRITLYLTEKKYSSCAWEVVRAEIMRSFSLSINLQKRLKSKE

SEQ ID NO: 7 - protein, 166 aa, Homo sapiens
CDLPQTHSLGNRRALILLGQMGRISPFSCLKDRHDFRIPQEEFDGNQFQKAQAISVLHEMIQQTFNLFSTEDSSAAWEQSLLEKFSTELYQQLNDLEACVIQEVGVEETPLMNEDSILAVRKYFQRITLYLIERKYSPCAWEVVRAEIMRSLSFSTNLQKRLRRKD

SEQ ID NO: 8 - protein, 166 aa, Homo sapiens
CDLPETHSLDNRRTLMLLAQMSRISPSSCLMDRHDFGFPQEEFDGNQFQKAPAISVLHELIQQIFNLFTTKDSSAAWDEDLLDKFCTELYQQLNDLEACVMQEERVGETPLMNVDSILAVKKYFRRITLYLTEKKYSPCAWEVVRAEIMRSLSLSTNLQERLRRKE

SEQ ID NO: 9 - protein, 166 aa, Homo sapiens
CDLPQTHSLGNRRALILLAQMGRISPFSCLKDRHDFGFPQEEFDGNQFQKAQAISVLHEMIQQTFNLFSTKDSSATWEQSLLEKFSTELNQQLNDMEACVIQEVGVEETPLMNVDSILAVKKYFQRITLYLTEKKYSPCAWEVVRAEIMRSFSLSKIFQERLRRKE

SEQ ID NO: 10 - protein, 166 aa, Homo sapiens
CDLPQTHSLSNRRTLMIMAQMGRISPFSCLKDRHDFGFPQEEFDGNQFQKAQAISVLHEMIQQTFNLFSTKDSSATWDETLLDKFYTELYQQLNDLEACMMQEVGVEDTPLMNVDSILTVRKYFQRITLYLTEKKYSPCAWEVVRAEIMRSFSLSANLQERLRRKE

SEQ ID NO: 11 - protein, 166 aa, Homo sapiens
CNLSQTHSLNNRRTLMLMAQMRRISPFSCLKDRHDFEFPQEEFDGNQFQKAQAISVLHEMMQQTFNLFSTKNSSAAWDETLLEKFYIELFQQMNDLEACVIQEVGVEETPLMNEDSILAVKKYFQRITLYLMEKKYSPCAWEVVRAEIMRSLSFSTNLQKRLRRKD

SEQ ID NO: 12 - protein, 166 aa, Homo sapiens
CDLPQTHSLGNRRALILLAQMGRISPFSCLKDRPDFGLPQEEFDGNQFQKTQAISVLHEMIQQTFNLFSTEDSSAAWEQSLLEKFSTELYQQLNNLEACVIQEVGMEETPLMNEDSILAVRKYFQRITLYLTEKKYSPCAWEVVRAEIMRSLSFSTNLQKILRRKD

SEQ ID NO: 13 - protein, 166 aa, Homo sapiens
CDLPQTHSLRNRRALILLAQMGRISPFSCLKDRHEFRFPEEEFDGHQFQKTQAISVLHEMIQQTFNLFSTEDSSAAWEQSLLEKFSTELYQQLNDLEACVIQEVGVEETPLMNEDFILAVRKYFQRITLYLMEKKYSPCAWEVVRAEIMRSFSFSTNLKKGLRRKD

SEQ ID NO: 14 - protein, 166 aa, Homo sapiens
CDLPQTHSLGHRRTMMLLAQMRRISLFSCLKDRHDFRFPQEEFDGNQFQKAEAISVLHEVIQQTFNLFSTKDSSVAWDERLLDKLYTELYQQLNDLEACVMQEVWVGGTPLMNEDSILAVRKYFQRITLYLTEKKYSPCAWEVVRAEIMRSFSSSRNLQERLRRKE

SEQ ID NO: 15 - protein, 166 aa, Homo sapiens
CDLPQTHSLGNRRALILLAQMGRISHFSCLKDRHDFGFPEEEFDGHQFQKTQAISVLHEMIQQTFNLFSTEDSSAAWEQSLLEKFSTELYQQLNDLEACVIQEVGVEETPLMNVDSILAVRKYFQRITLYLTEKKYSPCAWEVVRAEIMRSLSFSTNLQKRLRRKD

SEQ ID NO: 16 - protein, 166 aa, Homo sapiens
CDLPQTHSLGNRRALILLAQMGRISHFSCLKDRYDFGFPQEVFDGNQFQKAQAISAFHEMIQQTFNLFSTKDSSAAWDETLLDKFYIELFQQLNDLEACVTQEVGVEEIALMNEDSILAVRKYFQRITLYLMGKKYSPCAWEVVRAEIMRSFSFSTNLQKGLRRKD

SEQ ID NO: 17 - protein, 165 aa, Homo sapiens [sequence omitted]

SEQ ID NO: 18 - protein, 166 aa, Homo sapiens
CDLPETHSLDNRRTLMLLAQMSRISPSSCLMDRHDFGFPQEEFDGNQFQKAPAISVLHELIQQIFNLFTTKDSSAAWDEDLLDKFCTELYQQLNDLEACVMQEERVGETPLMNADSILAVKKYFRRITLYLTEKKYSPCAWEVVRAEIMRSLSLSTNLQERLRRKE

SEQ ID NO: 19 - protein, 166 aa, Homo sapiens
CDLPQTHSLGNRRALILLAQMGRISHFSCLKDRHDFGFPEEEFDGHQFQKAQAISVLHEMIQQTFNLFSTEDSSAAWEQSLLEKFSTELYQQLNDLEACVIQEVGVEETPLMNEDSILAVRKYFQRITLYLTEKKYSPCAWEVVRAEIMRSLSFSTNLQKRLRRKD

SEQ ID NO: 20 - protein, 166 aa, Homo sapiens
MSYNLLGFLQRSSNFQCQKLLWQLNGRLEYCLKDRMNFDIPEEIKQLQQFQKEDAALTIYEMLQNIFAIFRQDSSSTGWNETIVENLLANVYHQINHLKTVLEEKLEKEDFTRGKLMSSLHLKRYYGRILHYLKAKEYSHCAWTIVRVEILRNFYFINRLTGYLRN

SEQ ID NO: 21 - protein, 23 aa, Artificial Sequence
  Description of Artificial Sequence: Synthetic peptide
MALTFYLLVALVVLSYKSFSSLG

SEQ ID NO: 22 - protein, 23 aa, Artificial Sequence
  Description of Artificial Sequence: Synthetic peptide
MARSFSLLMVVLVLSYKSICSLG

SEQ ID NO: 23 - protein, 23 aa, Artificial Sequence
  Description of Artificial Sequence: Synthetic peptide
MALPFALLMALVVLSCKSSCSLD

SEQ ID NO: 24 - protein, 23 aa, Artificial Sequence
  Description of Artificial Sequence: Synthetic peptide
MALSFSLLMAVLVLSYKSICSLG

SEQ ID NO: 25 - protein, 23 aa, Artificial Sequence
  Description of Artificial Sequence: Synthetic peptide
MALTFALLVALLVLSCKSSCSVG

SEQ ID NO: 26 - protein, 557 aa, Homo sapiens
MMVVLLGATTLVLVAVAPWVLSAAAGGKNLKSPQKVEVDIIDDNFILRWNRSDESVGNVTFSFDYQKTGMDNWIKLSGCQNITSTKCNFSSLKLNVYEEIKLRIRAEKENTSSWYEVDSFTPFRKAQIGPPEVHLEAEDKAIVIHISPGTKDSVMWALDGLSFTYSLVIWKNSSGVEERIENIYSRHKIYKLSPETTYCLKVKAALLTSWKIGVYSPVHCIKTTVENELPPPENIEVSVQNQNYVLKWDYTYANMTFQVQWLHAFLKRNPGNHLYKWKQIPDCENVKTTQCVFPQNVFQKGIYLLRVQASDGNNTSFWSEEIKFDTEIQAFLLPPVFNIRSLSDSFHIYIGAPKQSGNTPVIQDYPLIYEIIFWENTSNAERKIIEKKTDVTVPNLKPLTVYCVKARAHTMDEKLNKSSVFSDAVCEKTKPGNTSKIWLIVGICIALFALPFVIYAAKVFLRCINYVFFPSLKPSSSIDEYFSEQPLKNLLLSTSEEQIEKCFIIENISTIATVEETNQTDEDHKKYSSQTSQDSGNYSNEDESESKTSEELQQDFV

SEQ ID NO: 27 - protein, 331 aa, Homo sapiens
MLLSQNAFIFRSLNLVLMVYISLVFGISYDSPDYTDESCTFKISLRNFRSILSWELKNHSIVPTHYTLLYTIMSKPEDLKVVKNCANTTRSFCDLTDEWRSTHEAYVTVLEGFSGNTTLFSCSHNFWLAIDMSFEPPEFEIVGFTNHINVMVKFPSIVEEELQFDLSLVIEEQSEGIVKKHKPEIKGNMSGNFTYIIDKLIPNTNYCVSVYLEHSDEQAVIKSPLKCTLLPPGQESESAESAKIGGIITVFLIALVLTSTIVTLKWIGYICLRNSLPKVLRQGLAKGWNAVAIHRCSHNALQSETPELKQSSCLSFPSSWDYKRASLCPSD

SEQ ID NO: 28 - protein, 121 aa, Artificial Sequence
  Description of Artificial Sequence: Synthetic polypeptide
EVQLVQSGAEVKKPGESLKISCKGSGYSFTSYWIGWVRQMPGKGLEWMGIIDPSDSDTRYSPSFQGQVTISADKSISTAYLQWSSLKASDTAMYYCARHPGLNWAPDFDYWGQGTLVTVSS

SEQ ID NO: 29 - protein, 107 aa, Artificial Sequence [sequence omitted]

SEQ ID NO: 30 - protein, 121 aa, Artificial Sequence
  Description of Artificial Sequence: Synthetic polypeptide
EVQLVQSGAEVKKPGESLKISCKGSGYSFTSYWIGWVRQMPGKGLEWMGIIDPSDSDTAYSPSFQGQVTISADKSISTAYLQWSSLKASDTAMYYCARHPGLNWAPDFDYWGQGTLVTVSS

SEQ ID NO: 31 - protein, 121 aa, Artificial Sequence
  Description of Artificial Sequence: Synthetic polypeptide
EVQLVQSGAEVKKPGESLKISCKGSGYSFTSYWIGWVRQMPGKGLEWMGIIDPSDSDTRYSPSFQGQVTISADKSISTAYLQWSSLKASDTAMYYCARHPGLAWAPDFDYWGQGTLVTVSS

SEQ ID NO: 32 - protein, 107 aa, Artificial Sequence
  Description of Artificial Sequence: Synthetic polypeptide
DIQMTQSPSSLSASVGDRVTITCRASQSIDGSLNWYQQKPGKAPKLLIYFASSLQSGVPSRFSGSGSGTDFTLTISSLQPEDFATYYCQQSYDFPLTFGQGTKVEIK

SEQ ID NO: 33 - protein, 107 aa, Artificial Sequence
  Description of Artificial Sequence: Synthetic polypeptide
DIQMTQSPSSLSASVGDRVTITCRASQSINRFLNWYQQKPGKAPKLLIYAASSLQSGVPSRFSGSGSGTDFTLTISSLQPEDFATYYCQQAIDLPFTFGQGTKVEIK

SEQ ID NO: 34 - protein, 107 aa, Artificial Sequence
  Description of Artificial Sequence: Synthetic polypeptide
DIQMTQSPSSLSASVGDRVTITCRASQSIGSFLNWYQQKPGKAPKLLIYFASSLQSGVPSRFSGSGSGTDFTLTISSLQPEDFATYYCQQSYSIPITFGQGTKVEIK

SEQ ID NO: 35 - protein, 107 aa, Artificial Sequence
  Description of Artificial Sequence: Synthetic polypeptide
DIQMTQSPSSLSASVGDRVTITCRASQSIGSALNWYQQKPGKAPKLLIYFASSLQSGVPSRFSGSGSGTDFTLTISSLQPEDFATYYCQQSYDFPLTFGQGTKVEIK

SEQ ID NO: 36 - protein, 107 aa, Artificial Sequence
  Description of Artificial Sequence: Synthetic polypeptide
DIQMTQSPSSLSASVGDRVTITCRASQSISKFLNWYQQKPGKAPKLLIYFASSLQSGVPSRFSGSGSGTDFTLTISSLQPEDFATYYCQQSNTLPFTFGQGTKVEIK

SEQ ID NO: 37 - protein, 107 aa, Artificial Sequence
  Description of Artificial Sequence: Synthetic polypeptide
DIQMTQSPSSLSASVGDRVTITCRASQSIDEFLNWYQQKPGKAPKLLIYFASSLQSGVPSRFSGSGSGTDFTLTISSLQPEDFATYYCQQAHSFPLTFGQGTKVEIK

SEQ ID NO: 38 - protein, 107 aa, Artificial Sequence
  Description of Artificial Sequence: Synthetic polypeptide
DIQMTQSPSSLSASVGDRVTITCRASQSITNFLNWYQQKPGKAPKLLIYFASSLQSGVPSRFSGSGSGTDFTLTISSLQPEDFATYYCQQSLDFPLTFGQGTKVEIK

SEQ ID NO: 39 - protein, 107 aa, Artificial Sequence
  Description of Artificial Sequence: Synthetic polypeptide
DIQMTQSPSSLSASVGDRVTITCRASQSIGDFLNWYQQKPGKAPKLLIYFASSLQSGVPSRFSGSGSGTDFTLTISSLQPEDFATYYCQQALDFPLTFGQGTKVEIK

SEQ ID NO: 40 - protein, 107 aa, Artificial Sequence
  Description of Artificial Sequence: Synthetic polypeptide
DIQMTQSPSSLSASVGDRVTITCRASQSIAEFLNWYQQKPGKAPKLLIYFASSLQSGVPSRFSGSGSGTDFTLTISSLQPEDFATYYCQQSIDFPLTFGQGTKVEIK

SEQ ID NO: 41 - protein, 107 aa, Artificial Sequence
  Description of Artificial Sequence: Synthetic polypeptide
DIQMTQSPSSLSASVGDRVTITCRASQSIGGFLNWYQQKPGKAPKLLIYFASSLQSGVPSRFSGSGSGTDFTLTISSLQPEDFATYYCQQSYSLPITFGQGTKVEIK

SEQ ID NO: 42 - protein, 107 aa, Artificial Sequence
  Description of Artificial Sequence: Synthetic polypeptide
DIQMTQSPSSLSASVGDRVTITCRASQSIGKSLNWYQQKPGKAPKLLIYFASSLQSGVPSRFSGSGSGTDFTLTISSLQPEDFATYYCQQSYDFPLTFGQGTKVEIK

SEQ ID NO: 43 - protein, 107 aa, Artificial Sequence
  Description of Artificial Sequence: Synthetic polypeptide
DIQMTQSPSSLSASVGDRVTITCRASQSIDDFLNWYQQKPGKAPKLLIYFASSLQSGVPSRFSGSGSGTDFTLTISSLQPEDFATYYCQQSHTLPLTFGQGTKVEIK

SEQ ID NO: 44 - protein, 107 aa, Artificial Sequence
  Description of Artificial Sequence: Synthetic polypeptide
DIQMTQSPSSLSASVGDRVTITCRASQSIDGALNWYQQKPGKAPKLLIYFASSLQSGVPSRFSGSGSGTDFTLTISSLQPEDFATYYCQQSFDFPLTFGQGTKVEIK

SEQ ID NO: 45 - protein, 107 aa, Artificial Sequence
  Description of Artificial Sequence: Synthetic polypeptide
DIQMTQSPSSLSASVGDRVTITCRASQSINNFLNWYQQKPGKAPKLLIYFASSLQSGVPSRFSGSGSGTDFTLTISSLQPEDFATYYCQQSFNLPITFGQGTKVEIK

SEQ ID NO: 46 - protein, 107 aa, Artificial Sequence
  Description of Artificial Sequence: Synthetic polypeptide
DIQMTQSPSSLSASVGDRVTITCRASQSIDRALNWYQQKPGKAPKLLIYFASSLQSGVPSRFSGSGSGTDFTLTISSLQPEDFATYYCQQSFDFPLTFGQGTKVEIK

SEQ ID NO: 47 - protein, 107 aa, Artificial Sequence
  Description of Artificial Sequence: Synthetic polypeptide
DIQMTQSPSSLSASVGDRVTITCRASQSITSSLNWYQQKPGKAPKLLIYFASSLQSGVPSRFSGSGSGTDFTLTISSLQPEDFATYYCQQSFDLPLTFGQGTKVEIK

SEQ ID NO: 48 - protein, 107 aa, Artificial Sequence
  Description of Artificial Sequence: Synthetic polypeptide
DIQMTQSPSSLSASVGDRVTITCRASQSINEFLNWYQQKPGKAPKLLIYFASSLQSGVPSRFSGSGSGTDFTLTISSLQPEDFATYYCQQSYSTPLTFGQGTKVEIK

SEQ ID NO: 49 - protein, 107 aa, Artificial Sequence
  Description of Artificial Sequence: Synthetic polypeptide
DIQMTQSPSSLSASVGDRVTITCRASQSISKFLNWYQQKPGKAPKLLIYFASSLQSGVPSRFSGSGSGTDFTLTISSLQPEDFATYYCQQSYDFPITFGQGTKVEIK

SEQ ID NO: 50 - protein, 107 aa, Artificial Sequence
  Description of Artificial Sequence: Synthetic polypeptide
DIQMTQSPSSLSASVGDRVTITCRASQSISEYLNWYQQKPGKAPKLLIYFASSLQSGVPSRFSGSGSGTDFTLTISSLQPEDFATYYCQQSHSLPITFGQGTKVEIK

SEQ ID NO: 51 - protein, 107 aa, Artificial Sequence
  Description of Artificial Sequence: Synthetic polypeptide
DIQMTQSPSSLSASVGDRVTITCRASQSITGFLNWYQQKPGKAPKLLIYAASSLQSGVPSRFSGSGSGTDFTLTISSLQPEDFATYYCQQSHDFPLTFGQGTKVEIK

SEQ ID NO: 52 - protein, 107 aa, Artificial Sequence
  Description of Artificial Sequence: Synthetic polypeptide
DIQMTQSPSSLSASVGDRVTITCRASQSINGVLNWYQQKPGKAPKLLIYFASSLQSGVPSRFSGSGSGTDFTLTISSLQPEDFATYYCQQSHDFPLTFGQGTKVEIK

SEQ ID NO: 53 - protein, 107 aa, Artificial Sequence
  Description of Artificial Sequence: Synthetic polypeptide
DIQMTQSPSSLSASVGDRVTITCRASQSIDGALNWYQQKPGKAPKLLIYFASSLQSGVPSRFSGSGSGTDFTLTISSLQPEDFATYYCQQAYDFPLTFGQGTKVEIK

SEQ ID NO: 54 - protein, 107 aa, Artificial Sequence
  Description of Artificial Sequence: Synthetic polypeptide
DIQMTQSPSSLSASVGDRVTITCRASQSIADFLNWYQQKPGKAPKLLIYFASSLQSGVPSRFSGSGSGTDFTLTISSLQPEDFATYYCQQSHSFPLTFGQGTKVEIK

SEQ ID NO: 55 - protein, 107 aa, Artificial Sequence
  Description of Artificial Sequence: Synthetic polypeptide
DIQMTQSPSSLSASVGDRVTITCRASQSITNHLNWYQQKPGKAPKLLIYFASSLQSGVPSRFSGSGSGTDFTLTISSLQPEDFATYYCQQAHNFPLTFGQGTKVEIK

SEQ ID NO: 56 - protein, 107 aa, Artificial Sequence
  Description of Artificial Sequence: Synthetic polypeptide
DIQMTQSPSSLSASVGDRVTITCRASQSIRNSLNWYQQKPGKAPKLLIKWASSLQSGVPSRFSGSGSGTDFTLTISSLQPEDFATYYCQQLYDWPLTFGQGTKVEIK

SEQ ID NO: 57 - protein, 108 aa, Artificial Sequence
  Description of Artificial Sequence: Synthetic polypeptide
DIQMTQSPSSLSASVGDRVTITCRASQSIANNNLNWYQQKPGKAPKLLIHWASSLQSGVPSRFSGSGSGTDFTLTISSLQPEDFATYYCQQGYDTPFTFGQGTKVEIK

SEQ ID NO: 58 - protein, 106 aa, Artificial Sequence
  Description of Artificial Sequence: Synthetic polypeptide
DIQMTQSPSSLSASVGDRVTITCRASQSINNLNWYQQKPGKAPKLLIYWASSLQSGVPSRFSGSGSGTDFTLTISSLQPEDFATYYCQQGYDTPFTFGQGTKVEIK

SEQ ID NO: 59 - protein, 108 aa, Artificial Sequence
  Description of Artificial Sequence: Synthetic polypeptide
DIQMTQSPSSLSASVGDRVTITCRASQSIRNNNLNWYQQKPGKAPKLLIHWASSLQSGVPSRFSGSGSGTDFTLTISSLQPEDFATYYCQQGYDTPFTFGQGTKVEIK

SEQ ID NO: 60 - protein, 108 aa, Artificial Sequence
  Description of Artificial Sequence: Synthetic polypeptide
DIQMTQSPSSLSASVGDRVTITCRASQSIRNNSLNWYQQKPGKAPKLLIYGASSLQSGVPSRFSGSGSGTDFTLTISSLQPEDFATYYCQQDYNWPITFGQGTKVEIK

SEQ ID NO: 61 - protein, 108 aa, Artificial Sequence
  Description of Artificial Sequence: Synthetic polypeptide
DIQMTQSPSSLSASVGDRVTITCRASQSIDNSYLNWYQQKPGKAPKLLIYGASSLQSGVPSRFSGSGSGTDFTLTISSLQPEDFATYYCQQGWDWPLTFGQGTKVEIK

SEQ ID NO: 62 - protein, 108 aa, Artificial Sequence
  Description of Artificial Sequence: Synthetic polypeptide
DIQMTQSPSSLSASVGDRVTITCRASQSIANTNLNWYQQKPGKAPKLLIHWASSLQSGVPSRFSGSGSGTDFTLTISSLQPEDFATYYCQQWYDNPLTFGQGTKVEIK

SEQ ID NO: 63 - protein, 108 aa, Artificial Sequence
  Description of Artificial Sequence: Synthetic polypeptide
DIQMTQSPSSLSASVGDRVTITCRASQSIDNNNLNWYQQKPGKAPKLLIYAASSLQSGVPSRFSGSGSGTDFTLTISSLQPEDFATYYCQQGYDWPLTFGQGTKVEIK

SEQ ID NO: 64 - protein, 108 aa, Artificial Sequence
  Description of Artificial Sequence: Synthetic polypeptide
DIQMTQSPSSLSASVGDRVTITCRASQSIRNNSLNWYQQKPGKAPKLLIYAASSLQSGVPSRFSGSGSGTDFTLTISSLQPEDFATYYCQQDYNWPLTFGQGTKVEIK

SEQ ID NO: 65 - protein, 106 aa, Artificial Sequence
  Description of Artificial Sequence: Synthetic polypeptide
DIQMTQSPSSLSASVGDRVTITCRASQSINYLNWYQQKPGKAPKLLIYGASSLQSGVPSRFSGSGSGTDFTLTISSLQPEDFATYYCQQSHDWPITFGQGTKVEIK

SEQ ID NO: 66 - protein, 108 aa, Artificial Sequence
  Description of Artificial Sequence: Synthetic polypeptide
DIQMTQSPSSLSASVGDRVTITCRASQSIRNNYLNWYQQKPGKAPKLLIYAASSLQSGVPSRFSGSGSGTDFTLTISSLQPEDFATYYCQQGYDTPLTFGQGTKVEIK

SEQ ID NO: 67 - protein, 108 aa, Artificial Sequence
  Description of Artificial Sequence: Synthetic polypeptide
DIQMTQSPSSLSASVGDRVTITCRASQSISNSNLNWYQQKPGKAPKLLIHWASSLQSGVPSRFSGSGSGTDFTLTISSLQPEDFATYYCQQWYDHPLTFGQGTKVEIK

SEQ ID NO: 68 - protein, 108 aa, Artificial Sequence
  Description of Artificial Sequence: Synthetic polypeptide
DIQMTQSPSSLSASVGDRVTITCRASQSIRNTNLNWYQQKPGKAPKLLIHWASSLQSGVPSRFSGSGSGTDFTLTISSLQPEDFATYYCQQGYDTPFTFGQGTKVEIK

SEQ ID NO: 69 - protein, 108 aa, Artificial Sequence
  Description of Artificial Sequence: Synthetic polypeptide
DIQMTQSPSSLSASVGDRVTITCRASQSIANNDLNWYQQKPGKAPKLLIHWASSLQSGVPSRFSGSGSGTDFTLTISSLQPEDFATYYCQQDYDWPLTFGQGTKVEIK

SEQ ID NO: 70 - protein, 107 aa, Artificial Sequence
  Description of Artificial Sequence: Synthetic polypeptide
DIQMTQSPSSLSASVGDRVTITCRASQSIAGFLNWYQQKPGKAPKLLIYYASSLQSGVPSRFSGSGSGTDFTLTISSLQPEDFATYYCQQSYSIPITFGQGTKVEIK

SEQ ID NO: 71 - protein, 107 aa, Artificial Sequence
  Description of Artificial Sequence: Synthetic polypeptide
DIQMTQSPSSLSASVGDRVTITCRASQSIDGFLNWYQQKPGKAPKLLIYFASSLQSGVPSRFSGSGSGTDFTLTISSLQPEDFATYYCQQSYDLPITFGQGTKVEIK

SEQ ID NO: 72 - DNA, 321 bp, Artificial Sequence
  Description of Artificial Sequence: Synthetic polynucleotide
gatattcagatgacccagagcccgagcagcctgagcgcgagcgtgggcgatcgcgtgaccattacctgccgcgcgagccagagcattgatgggttcctgaactggtatcagcagaaaccgggcaaagcgccgaaactgctgatttatttcgcgagcagcctgcagagcggcgtgccgagccgctttagcggcagcggcagcggcaccgattttaccctgaccattagcagcctgcagccggaagattttgcgacctattattgccagcagtcctacgacctcccgattacatttggccagggcaccaaagtggaaattaaa

SEQ ID NO: 73 - protein, 107 aa, Artificial Sequence
  Description of Artificial Sequence: Synthetic polypeptide
DIQMTQSPSSLSASVGDRVTITCRASQSIEGALNWYQQKPGKAPKLLIYFASSLQSGVPSRFSGSGSGTDFTLTISSLQPEDFATYYCQQAYDFPLTFGQGTKVEIK

SEQ ID NO: 74 - protein, 107 aa, Artificial Sequence
  Description of Artificial Sequence: Synthetic polypeptide
DIQMTQSPSSLSASVGDRVTITCRASQSIEGYLNWYQQKPGKAPKLLIYFASSLQSGVPSRFSGSGSGTDFTLTISSLQPEDFATYYCQQAYDFPLTFGQGTKVEIK

SEQ ID NO: 75 - protein, 107 aa, Artificial Sequence
  Description of Artificial Sequence: Synthetic polypeptide
DIQMTQSPSSLSASVGDRVTITCRASQSISSALNWYQQKPGKAPKLLIYFASSLQSGVPSRFSGSGSGTDFTLTISSLQPEDFATYYCQQAYDFPLTFGQGTKVEIK

SEQ ID NO: 76 - protein, 6 aa, Artificial Sequence
  Description of Artificial Sequence: Synthetic peptide
QSIADF

SEQ ID NO: 77 - protein, 6 aa, Artificial Sequence
  Description of Artificial Sequence: Synthetic peptide
QSIAEF

SEQ ID NO: 78 - protein, 7 aa, Artificial Sequence
  Description of Artificial Sequence: Synthetic peptide
QSIANNN

SEQ ID NO: 79 - protein, 7 aa, Artificial Sequence
  Description of Artificial Sequence: Synthetic peptide
QSIANTN

SEQ ID NO: 80 - protein, 6 aa, Artificial Sequence
  Description of Artificial Sequence: Synthetic peptide
QSIDGA

SEQ ID NO: 81 - protein, 6 aa, Artificial Sequence
  Description of Artificial Sequence: Synthetic peptide
QSIDGF

SEQ ID NO: 82 - protein, 7 aa, Artificial Sequence
  Description of Artificial Sequence: Synthetic peptide
QSIDNSY

SEQ ID NO: 83 - protein, 6 aa, Artificial Sequence
  Description of Artificial Sequence: Synthetic peptide
QSIDRA

SEQ ID NO: 84 - protein, 6 aa, Artificial Sequence
  Description of Artificial Sequence: Synthetic peptide
QSIEGA

SEQ ID NO: 85 - protein, 6 aa, Artificial Sequence
  Description of Artificial Sequence: Synthetic peptide
QSIGDF

SEQ ID NO: 86 - protein, 6 aa, Artificial Sequence
  Description of Artificial Sequence: Synthetic peptide
QSIGKS

SEQ ID NO: 87 - protein, 6 aa, Artificial Sequence
  Description of Artificial Sequence: Synthetic peptide
QSIGSA

SEQ ID NO: 88 - protein, 6 aa, Artificial Sequence
  Description of Artificial Sequence: Synthetic peptide
QSINGV

SEQ ID NO: 89 - protein, 7 aa, Artificial Sequence
  Description of Artificial Sequence: Synthetic peptide
QSIRNTN

SEQ ID NO: 90 - protein, 6 aa, Artificial Sequence
  Description of Artificial Sequence: Synthetic peptide
QSISSA

SEQ ID NO: 91 - protein, 6 aa, Artificial Sequence
  Description of Artificial Sequence: Synthetic peptide
QSISSF

SEQ ID NO: 92 - DNA, 324 bp, Artificial Sequence
  Description of Artificial Sequence: Synthetic polynucleotide
gacatccaaatgacgcagtctccgagctctctgagcgcatccgtgggcgatcgcgtaactatcacttgtcgcgcctcccagagcattgataactcctatctcaattggtatcaacaaaaaccgggtaaggcaccgaaactgctgatttacggagcgtcctctctgcagtccggtgtgccgtcccgtttctccggcagcggttctggtaccgatttcacgctgaccatcagctctctgcaaccggaggactttgctacgtactactgccaacagggctacgatttccctctcacattcggccaaggtaccaaagtggaaattaaa

SEQ ID NO: 93 - protein, 3 aa, Artificial Sequence
  Description of Artificial Sequence: Synthetic peptide
FAS

SEQ ID NO: 94 - protein, 3 aa, Artificial Sequence
  Description of Artificial Sequence: Synthetic peptide
GAS

SEQ ID NO: 95 - protein, 3 aa, Artificial Sequence
  Description of Artificial Sequence: Synthetic peptide
WAS

SEQ ID NO: 96 - protein, 9 aa, Artificial Sequence
  Description of Artificial Sequence: Synthetic peptide
QQALDFPLT

SEQ ID NO: 97 - protein, 9 aa, Artificial Sequence
  Description of Artificial Sequence: Synthetic peptide
QQAYDFPLT

SEQ ID NO: 98 - protein, 9 aa, Artificial Sequence
  Description of Artificial Sequence: Synthetic peptide
QQGWDWPLT

SEQ ID NO: 99 - protein, 9 aa, Artificial Sequence
  Description of Artificial Sequence: Synthetic peptide
QQGYDFPLT

SEQ ID NO: 100 - protein, 9 aa, Artificial Sequence
  Description of Artificial Sequence: Synthetic peptide
QQGYDTPFT

SEQ ID NO: 101 - protein, 9 aa, Artificial Sequence
  Description of Artificial Sequence: Synthetic peptide
QQSFDFPLT

SEQ ID NO: 102 - protein, 9 aa, Artificial Sequence
  Description of Artificial Sequence: Synthetic peptide
QQSHDFPLT

SEQ ID NO: 103 - protein, 9 aa, Artificial Sequence
  Description of Artificial Sequence: Synthetic peptide
QQSHSFPLT

SEQ ID NO: 104 - protein, 9 aa, Artificial Sequence
  Description of Artificial Sequence: Synthetic peptide
QQSIDFPLT

SEQ ID NO: 105 - protein, 9 aa, Artificial Sequence
  Description of Artificial Sequence: Synthetic peptide
QQSYDFPLT

SEQ ID NO: 106 - protein, 9 aa, Artificial Sequence
  Description of Artificial Sequence: Synthetic peptide
QQSYDLPIT

SEQ ID NO: 107 - protein, 9 aa, Artificial Sequence
  Description of Artificial Sequence: Synthetic peptide
QQWYDNPLT

SEQ ID NO: 108 - DNA, 321 bp, Artificial Sequence
  Description of Artificial Sequence: Synthetic polynucleotide
gatattcagatgacccagagcccgagcagcctgagcgcgagcgtgggcgatcgcgtgaccattacctgccgcgcgagccagagcatcgatggcgccctgaactggtatcagcagaaaccgggcaaagcgccgaaactgctgatttatttcgcgagcagcctgcagagcggcgtgccgagccgctttagcggcagcggcagcggcaccgattttaccctgaccattagcagcctgcagccggaagattttgcgacctattattgccagcaggcctacgactttccgttgacatttggccagggcaccaaagtggaaattaaa

SEQ ID NO: 109 - protein, 8 aa, Artificial Sequence
  Description of Artificial Sequence: Synthetic peptide
GYSFTSYW

SEQ ID NO: 110 - DNA, 363 bp, Artificial Sequence
  Description of Artificial Sequence: Synthetic polynucleotide
gaggtgcagctggtgcagagcggcgccgaggtgaagaagcccggcgagagcctgaagatcagctgcaagggcagcggctacagcttcaccagctactggatcggctgggtgcggcagatgcccggcaagggcctggagtggatgggcatcatcgaccccagcgacagcgacacccggtacagccccagcttccagggccaggtgaccatcagcgccgacaagagcatcagcaccgcctacctgcagtggagcagcctgaaggccagcgacaccgccatgtactactgcgcccggcaccccggcctgaactgggcccccgacttcgactactggggccagggcaccctggtgaccgtgagcagc

SEQ ID NO: 111 - protein, 8 aa, Artificial Sequence
  Description of Artificial Sequence: Synthetic peptide
IAPSDSDT

SEQ ID NO: 112 - protein, 8 aa, Artificial Sequence
  Description of Artificial Sequence: Synthetic peptide
IDASDSDT

SEQ ID NO: 113 - protein, 8 aa, Artificial Sequence
  Description of Artificial Sequence: Synthetic peptide
IDPSDSDT

SEQ ID NO: 114 - protein, 8 aa, Artificial Sequence
  Description of Artificial Sequence: Synthetic peptide
  MOD_RES (2)..(2): Asp or Ala
  MOD_RES (3)..(3): Pro or Ala
IXXSDSDT

SEQ ID NO: 115 - protein, 14 aa, Artificial Sequence
  Description of Artificial Sequence: Synthetic peptide
ARHPGLAWAPDFDY

SEQ ID NO: 116 - protein, 14 aa, Artificial Sequence
  Description of Artificial Sequence: Synthetic peptide
ARHPGLNWAPDFDY

SEQ ID NO: 117 - DNA, 363 bp, Artificial Sequence
  Description of Artificial Sequence: Synthetic polynucleotide
gaggtgcagctggtgcagagcggcgccgaggtgaagaagcccggcgagagcctgaagatcagctgcaagggcagcggctacagcttcaccagctactggatcggctgggtgcggcagatgcccggcaagggcctggagtggatgggcatcatcgacgccagcgacagcgacacccggtacagccccagcttccagggccaggtgaccatcagcgccgacaagagcatcagcaccgcctacctgcagtggagcagcctgaaggccagcgacaccgccatgtactactgcgcccggcaccccggcctgaactgggcccccgacttcgactactggggccagggcaccctggtgaccgtgagcagc

SEQ ID NO: 118 - protein, 7 aa, Artificial Sequence
  Description of Artificial Sequence: Synthetic peptide
  MOD_RES (4)..(4): Gly, Asp, Ala, Arg, Glu, Ser or Asn
  MOD_RES (5)..(5): Asp, Gly, Asn, Ser, Arg, Glu or Lys
  MOD_RES (6)..(6): Phe, Ala, Asn, Thr, Ser or Val
  MOD_RES (7)..(7): Tyr, Asn or not present
QSIXXXX

SEQ ID NO: 119 - protein, 3 aa, Artificial Sequence
  Description of Artificial Sequence: Synthetic peptide
  MOD_RES (1)..(1): Phe, Trp or Gly
XAS

SEQ ID NO: 120 - protein, 9 aa, Artificial Sequence
  Description of Artificial Sequence: Synthetic peptide
  MOD_RES (3)..(3): Ala, Gly, Ser or Trp
  MOD_RES (4)..(4): Leu, Tyr, His, Trp, Phe or Ile
  MOD_RES (5)..(5): Asp or Ser
  MOD_RES (6)..(6): Phe, Thr, Leu, Asn or Trp
  MOD_RES (8)..(8): Leu, Phe or Ile
QQXXXXPXT

SEQ ID NO: 121 - protein, 14 aa, Artificial Sequence
  Description of Artificial Sequence: Synthetic peptide
  MOD_RES (7)..(7): Ala or Asn
ARHPGLXWAPDFDY

SEQ ID NO: 122 - DNA, 363 bp, Artificial Sequence
  Description of Artificial Sequence: Synthetic polynucleotide
gaggtgcagctggtgcagagcggcgccgaggtgaagaagcccggcgagagcctgaagatcagctgcaagggcagcggctacagcttcaccagctactggatcggctgggtgcggcagatgcccggcaagggcctggagtggatgggcatcatcgaccccagcgacagcgacacccggtacagccccagcttccagggccaggtgaccatcagcgccgacaagagcatcagcaccgcctacctgcagtggagcagcctgaaggccagcgacaccgccatgtactactgcgcccggcaccccggcctggcctgggcccccgacttcgactactggggccagggcaccctggtgaccgtgagcagc

SEQ ID NO: 123 - protein, 107 aa, Artificial Sequence
  Description of Artificial Sequence: Synthetic polypeptide
DIQMTQSPSSLSASVGDRVTITCRASQSISGFLNWYQQKPGKAPKLLIYFASSLQSGVPSRFSGSGSGTDFTLTISSLQPEDFATYYCQQSYDLPITFGQGTKVEIK

SEQ ID NO: 124 - protein, 107 aa, Artificial Sequence
  Description of Artificial Sequence: Synthetic polypeptide
DIQMTQSPSSLSASVGDRVTITCRASQSIEGFLNWYQQKPGKAPKLLIYFASSLQSGVPSRFSGSGSGTDFTLTISSLQPEDFATYYCQQSYDLPITFGQGTKVEIK

SEQ ID NO: 125 - protein, 107 aa, Artificial Sequence
  Description of Artificial Sequence: Synthetic polypeptide
DIQMTQSPSSLSASVGDRVTITCRASQSIDGYLNWYQQKPGKAPKLLIYFASSLQSGVPSRFSGSGSGTDFTLTISSLQPEDFATYYCQQSYDLPITFGQGTKVEIK

SEQ ID NO: 126 - protein, 107 aa, Artificial Sequence
  Description of Artificial Sequence: Synthetic polypeptide
DIQMTQSPSSLSASVGDRVTITCRASQSIDGFLNWYQQKPGKAPKLLIYAASSLQSGVPSRFSGSGSGTDFTLTISSLQPEDFATYYCQQSYDLPITFGQGTKVEIK

SEQ ID NO: 127 - protein, 107 aa, Artificial Sequence
  Description of Artificial Sequence: Synthetic polypeptide
DIQMTQSPSSLSASVGDRVTITCRASQSIDGFLNWYQQKPGKAPKLLIYIASSLQSGVPSRFSGSGSGTDFTLTISSLQPEDFATYYCQQSYDLPITFGQGTKVEIK

SEQ ID NO: 128 - protein, 107 aa, Artificial Sequence
  Description of Artificial Sequence: Synthetic polypeptide
DIQMTQSPSSLSASVGDRVTITCRASQSIDGFLNWYQQKPGKAPKLLIYLASSLQSGVPSRFSGSGSGTDFTLTISSLQPEDFATYYCQQSYDLPITFGQGTKVEIK

SEQ ID NO: 129 - protein, 107 aa, Artificial Sequence
  Description of Artificial Sequence: Synthetic polypeptide
DIQMTQSPSSLSASVGDRVTITCRASQSIDGFLNWYQQKPGKAPKLLIYVASSLQSGVPSRFSGSGSGTDFTLTISSLQPEDFATYYCQQSYDLPITFGQGTKVEIK

SEQ ID NO: 130 - protein, 107 aa, Artificial Sequence
  Description of Artificial Sequence: Synthetic polypeptide
DIQMTQSPSSLSASVGDRVTITCRASQSIEGYLNWYQQKPGKAPKLLIYFASSLQSGVPSRFSGSGSGTDFTLTISSLQPEDFATYYCQQSYDLPITFGQGTKVEIK

SEQ ID NO: 131 - protein, 107 aa, Artificial Sequence
  Description of Artificial Sequence: Synthetic polypeptide
DIQMTQSPSSLSASVGDRVTITCRASQSIEGFLNWYQQKPGKAPKLLIYAASSLQSGVPSRFSGSGSGTDFTLTISSLQPEDFATYYCQQSYDLPITFGQGTKVEIK

SEQ ID NO: 132 - protein, 107 aa, Artificial Sequence
  Description of Artificial Sequence: Synthetic polypeptide
DIQMTQSPSSLSASVGDRVTITCRASQSIEGFLNWYQQKPGKAPKLLIYIASSLQSGVPSRFSGSGSGTDFTLTISSLQPEDFATYYCQQSYDLPITFGQGTKVEIK

SEQ ID NO: 133 - protein, 107 aa, Artificial Sequence
  Description of Artificial Sequence: Synthetic polypeptide
DIQMTQSPSSLSASVGDRVTITCRASQSIEGFLNWYQQKPGKAPKLLIYLASSLQSGVPSRFSGSGSGTDFTLTISSLQPEDFATYYCQQSYDLPITFGQGTKVEIK

SEQ ID NO: 134 - protein, 107 aa, Artificial Sequence
  Description of Artificial Sequence: Synthetic polypeptide
DIQMTQSPSSLSASVGDRVTITCRASQSIEGFLNWYQQKPGKAPKLLIYVASSLQSGVPSRFSGSGSGTDFTLTISSLQPEDFATYYCQQSYDLPITFGQGTKVEIK

SEQ ID NO: 135 - protein, 107 aa, Artificial Sequence
  Description of Artificial Sequence: Synthetic polypeptide
DIQMTQSPSSLSASVGDRVTITCRASQSISSFLNWYQQKPGKAPKLLIYFASSLQSGVPSRFSGSGSGTDFTLTISSLQPEDFATYYCQQSYDLPITFGQGTKVEIK

SEQ ID NO: 136 - protein, 107 aa, Artificial Sequence
  Description of Artificial Sequence: Synthetic polypeptide
DIQMTQSPSSLSASVGDRVTITCRASQSISSYLNWYQQKPGKAPKLLIYFASSLQSGVPSRFSGSGSGTDFTLTISSLQPEDFATYYCQQSYDLPITFGQGTKVEIK

SEQ ID NO: 137 - protein, 107 aa, Artificial Sequence
  Description of Artificial Sequence: Synthetic polypeptide
DIQMTQSPSSLSASVGDRVTITCRASQSIGDFLNWYQQKPGKAPKLLIYYASSLQSGVPSRFSGSGSGTDFTLTISSLQPEDFATYYCQQSYDLPITFGQGTKVEIK

SEQ ID NO: 138 - protein, 107 aa, Artificial Sequence
  Description of Artificial Sequence: Synthetic polypeptide
DIQMTQSPSSLSASVGDRVTITCRASQSIEGYLNWYQQKPGKAPKLLIYYASSLQSGVPSRFSGSGSGTDFTLTISSLQPEDFATYYCQQSYDLPITFGQGTKVEIK

SEQ ID NO: 139 - protein, 107 aa, Artificial Sequence
  Description of Artificial Sequence: Synthetic polypeptide
DIQMTQSPSSLSASVGDRVTITCRASQSIEGFLNWYQQKPGKAPKLLIYYASSLQSGVPSRFSGSGSGTDFTLTISSLQPEDFATYYCQQSYDLPITFGQGTKVEIK

SEQ ID NO: 140 - protein, 107 aa, Artificial Sequence
  Description of Artificial Sequence: Synthetic polypeptide
DIQMTQSPSSLSASVGDRVTITCRASQSISSFLNWYQQKPGKAPKLLIYYASSLQSGVPSRFSGSGSGTDFTLTISSLQPEDFATYYCQQSYDLPITFGQGTKVEIK

SEQ ID NO: 141 - protein, 107 aa, Artificial Sequence
  Description of Artificial Sequence: Synthetic polypeptide
DIQMTQSPSSLSASVGDRVTITCRASQSISGALNWYQQKPGKAPKLLIYFASSLQSGVPSRFSGSGSGTDFTLTISSLQPEDFATYYCQQAYDFPLTFGQGTKVEIK

SEQ ID NO: 142 - protein, 107 aa, Artificial Sequence
  Description of Artificial Sequence: Synthetic polypeptide
DIQMTQSPSSLSASVGDRVTITCRASQSIDGYLNWYQQKPGKAPKLLIYFASSLQSGVPSRFSGSGSGTDFTLTISSLQPEDFATYYCQQAYDFPLTFGQGTKVEIK

SEQ ID NO: 143 - protein, 107 aa, Artificial Sequence
  Description of Artificial Sequence: Synthetic polypeptide
DIQMTQSPSSLSASVGDRVTITCRASQSIDGALNWYQQKPGKAPKLLIYFASSLQSGVPSRFSGSGSGTDFTLTISSLQPEDFATYYCQQAYDLPLTFGQGTKVEIK

SEQ ID NO: 144 - protein, 107 aa, Artificial Sequence
  Description of Artificial Sequence: Synthetic polypeptide
DIQMTQSPSSLSASVGDRVTITCRASQSISSYLNWYQQKPGKAPKLLIYFASSLQSGVPSRFSGSGSGTDFTLTISSLQPEDFATYYCQQAYDFPLTFGQGTKVEIK

SEQ ID NO: 145 - protein, 107 aa, Artificial Sequence
  Description of Artificial Sequence: Synthetic polypeptide
DIQMTQSPSSLSASVGDRVTITCRASQSISSALNWYQQKPGKAPKLLIYFASSLQSGVPSRFSGSGSGTDFTLTISSLQPEDFATYYCQQAYDLPLTFGQGTKVEIK

SEQ ID NO: 146 - protein, 107 aa, Artificial Sequence
  Description of Artificial Sequence: Synthetic polypeptide
DIQMTQSPSSLSASVGDRVTITCRASQSISSYLNWYQQKPGKAPKLLIYFASSLQSGVPSRFSGSGSGTDFTLTISSLQPEDFATYYCQQAYDLPLTFGQGTKVEIK

SEQ ID NO: 147 - protein, 107 aa, Artificial Sequence
  Description of Artificial Sequence: Synthetic polypeptide
DIQMTQSPSSLSASVGDRVTITCRASQSIGDFLNWYQQKPGKAPKLLIYAASSLQSGVPSRFSGSGSGTDFTLTISSLQPEDFATYYCQQAYDLPLTFGQGTKVEIK

SEQ ID NO: 148 - protein, 108 aa, Artificial Sequence
  Description of Artificial Sequence: Synthetic polypeptide
DIQMTQSPSSLSASVGDRVTITCRASQSIDNSYLNWYQQKPGKAPKLLIYGASSLQSGVPSRFSGSGSGTDFTLTISSLQPEDFATYYCQQGYDWPLTFGQGTKVEIK

SEQ ID NO: 149 - protein, 108 aa, Artificial Sequence
  Description of Artificial Sequence: Synthetic polypeptide
DIQMTQSPSSLSASVGDRVTITCRASQSIDNSYLNWYQQKPGKAPKLLIYGASSLQSGVPSRFSGSGSGTDFTLTISSLQPEDFATYYCQQGWDFPLTFGQGTKVEIK

SEQ ID NO: 150 - protein, 108 aa, Artificial Sequence
  Description of Artificial Sequence: Synthetic polypeptide
DIQMTQSPSSLSASVGDRVTITCRASQSIDNSYLNWYQQKPGKAPKLLIYGASSLQSGVPSRFSGSGSGTDFTLTISSLQPEDFATYYCQQGYDFPLTFGQGTKVEIK

SEQ ID NO: 151 - protein, 108 aa, Artificial Sequence
  Description of Artificial Sequence: Synthetic polypeptide
DIQMTQSPSSLSASVGDRVTITCRASQSIDQSYLNWYQQKPGKAPKLLIYGASSLQSGVPSRFSGSGSGTDFTLTISSLQPEDFATYYCQQGYDFPLTFGQGTKVEIK

SEQ ID NO: 152 - protein, 108 aa, Artificial Sequence
  Description of Artificial Sequence: Synthetic polypeptide
DIQMTQSPSSLSASVGDRVTITCRASQSIDTSYLNWYQQKPGKAPKLLIYGASSLQSGVPSRFSGSGSGTDFTLTISSLQPEDFATYYCQQGYDFPLTFGQGTKVEIK

SEQ ID NO: 153 - protein, 108 aa, Artificial Sequence
  Description of Artificial Sequence: Synthetic polypeptide
DIQMTQSPSSLSASVGDRVTITCRASQSIDNTYLNWYQQKPGKAPKLLIYGASSLQSGVPSRFSGSGSGTDFTLTISSLQPEDFATYYCQQGYDFPLTFGQGTKVEIK

SEQ ID NO: 154 - protein, 8 aa, Artificial Sequence
  Description of Artificial Sequence: Synthetic peptide
QQSYDFPL

SEQ ID NO: 155 - protein, 98 aa, Homo sapiens
EVQLVQSGAEVKKPGESLKISCKGSGYSFTSYWIGWVRQMPGKGLEWMGIIYPGDSDTRYSPSFQGQVTISADKSISTAYLQWSSLKASDTAVYYCAR

SEQ ID NO: 156 - protein, 107 aa, Homo sapiens
DIQMTQSPSSLSASVGDRVTITCRASQSISSYLNWYQQKPGKAPKLLIYAASSLQSGVPSRFSGSGSGTDFTLTISSLQPEDFATYYCQQSYSTPWTFGQGTKVEIK

SEQ ID NO: 157 - protein, 121 aa, Artificial Sequence
  Description of Artificial Sequence: Synthetic polypeptide
EVQLVQSGAEVKKPGESLKISCKGSGYSFTSYWIGWVRQMPGKGLEWMGIIAPSDSDTRYSPSFQGQVTISADKSISTAYLQWSSLKASDTAMYYCARHPGLNWAPDFDYWGQGTLVTVSS

SEQ ID NO: 158 - protein, 121 aa, Artificial Sequence
  Description of Artificial Sequence: Synthetic polypeptide
EVQLVQSGAEVKKPGESLKISCKGSGYSFTSYWIGWVRQMPGKGLEWMGIIDASDSDTRYSPSFQGQVTISADKSISTAYLQWSSLKASDTAMYYCARHPGLNWAPDFDYWGQGTLVTVSS

SEQ ID NO: 159 - protein, 7 aa, Artificial Sequence
  Description of Artificial Sequence: Synthetic peptide
  MOD_RES (4)..(4): Gly, Asp, Ala, Glu, Ser or Asn
  MOD_RES (5)..(5): Asp, Gly, Asn, Ser or Arg
  MOD_RES (6)..(6): Phe, Ala, Asn, Ser or Val
  MOD_RES (7)..(7): Tyr, Asn or not present
QSIXXXX

SEQ ID NO: 160 - protein, 9 aa, Artificial Sequence
  Description of Artificial Sequence: Synthetic peptide
  MOD_RES (3)..(3): Ala, Gly or Ser
  MOD_RES (4)..(4): Tyr, His, Trp or Phe
  MOD_RES (5)..(5): Asp or Ser
  MOD_RES (6)..(6): Phe, Thr, Leu or Trp
  MOD_RES (8)..(8): Leu, Phe or Ile
QQXXXXPXT

SEQ ID NO: 161 - protein, 7 aa, Artificial Sequence
  Description of Artificial Sequence: Synthetic peptide
  MOD_RES (4)..(4): Ala or Asp
  MOD_RES (5)..(5): Asn or Gly
  MOD_RES (6)..(6): Phe, Asn or Ser
  MOD_RES (7)..(7): Tyr, Asn or not present
QSIXXXX

SEQ ID NO: 162 - protein, 9 aa, Artificial Sequence
  Description of Artificial Sequence: Synthetic peptide
  MOD_RES (3)..(3): Gly or Ser
  MOD_RES (6)..(6): Phe, Thr or Leu
  MOD_RES (8)..(8): Leu, Phe or Ile
QQXYDXPXT